European Patent Specification EP 2 814 968 B1, published May 27, 2026. Title: Improving drought resistance in plants: pectinesterase. Applicant: Keygene N.V. The sequence listing filed with the application follows.

SEQUENCE LISTING (10 sequences)

SEQ ID NO: 1 - DNA, 1149 bp, Arabidopsis thaliana
atgcccaaactcaattcaacccaagctcccaatttattccttctccttctcgttatccttctttgttcaacgcaaacacaatgccacaccaaaggtctccgattacgaccaagaaaccagaagaatatgaacacgacgagtgatcggacacaaaacccggaagatgagttcatgaaatgggtgagattcgttggaagccttaaacactcagtgttcaaggcagccaagaacaaactcttcccttcttatacattaactgtccacaagaaatccaataaaggtgacttcactaaaatccaagacgccattgattctctccctctcatcaactttgttcgtgtcgtcatcaaagttcatgccggagtttacaaggagaaggtgagcatacccccactgaaggcatttataacaatagaaggagaaggagcagagaagacaacagtggaatggggagacacagcacaaacccctgactcaaaaggcaaccccatgggcacttacaactcggcctcgttcgcggtcaactctcctttctttgtcgctaagaatatcacattcaggaacacgaccccagtccccttgcccggtgcagttggtaaacaggcggtagcattgagggtgtcggcagacaatgccgcgttttttgggtgtagaatgcttggtgctcaagacactctctatgaccatttgggaagacattattacaaagattgttacattgagggatcagtggacttcatctttggaaatgccctttctctttatgaagggtgccacgtgcatgcgatagcggataagctaggagcagtgacggcacaggggaggagcagtgttctagaggacaccggattctcgttcgtaaagtgtaaggtgacagggacaggggttttgtatcttgggagggcatggggtcccttctcaagagtcgtttttgcttacacttacatggacaacatcatcctccctagaggctggtacaattggggagacccttcccgtgagatgacggtgttctatgggcagtacaagtgcacgggagcaggagcaaactatggagggagggtggcttgggcaagagagctcaccgacgaagaagctaagccttttctttctcttacctttatcgacggctctgaatggatcaaactc

SEQ ID NO: 2 - protein, 383 aa, Arabidopsis thaliana
MPKLNSTQAPNLFLLLLVILLCSTQTQCHTKGLRLRPRNQKNMNTTSDRTQNPEDEFMKWVRFVGSLKHSVFKAAKNKLFPSYTLTVHKKSNKGDFTKIQDAIDSLPLINFVRVVIKVHAGVYKEKVSIPPLKAFITIEGEGAEKTTVEWGDTAQTPDSKGNPMGTYNSASFAVNSPFFVAKNITFRNTTPVPLPGAVGKQAVALRVSADNAAFFGCRMLGAQDTLYDHLGRHYYKDCYIEGSVDFIFGNALSLYEGCHVHAIADKLGAVTAQGRSSVLEDTGFSFVKCKVTGTGVLYLGRAWGPFSRVVFAYTYMDNIILPRGWYNWGDPSREMTVFYGQYKCTGAGANYGGRVAWARELTDEEAKPFLSLTFIDGSEWIKL

SEQ ID NO: 3 - DNA, 1149 bp, Brassica rapa
atgccccaattcagttcatcccaagctcccattttaatcctccccgttctcattatacttctgtgttcaacgcaaacacaatgccacaccaaagggctacgattgcgaccaagaaaccagaagattgtgaactctacgagtcagacacaaaaccctgaagaggaattcttgaaatgggttagatacgttgggagccttaagcacacggtgttcaaggcagccaagaacaaactcttcgcttcgtatacactcactgttcataagaaacacaacaaaggtgacttcactaaaatccaagacgccatagattctctgcctctcatcaacctcgttcgtgtcgtcatcaaagttcatgctggagtttacaaggaaaaggtgaacatacctccaatgaaggcattcataacaatagaaggagaaggagcagataaaacaatagtgcaatggggagacacagcacaaacacatgacccaaaaggcaatcccatgggcaccttcaactctgcctcttttgccgtcaactctcctttctttgtcgcgaagaacatcactttcaagaacacgacaccagtccccttgccaggcgcggttggaaaacaagcggtggcattgagagtgtcagccgacaatgctgcttttttcgggtgtaaaatgcttggtgctcaagacactctctatgaccatttgggaagacattattacaaagactgttacattgaaggatccgttgatttcatctttggcaatgccctttctctctacgaggggtgtcacgtgcacgcaatagcggataagctaggagcagtgacggcgcaaggaaggagcagtgtgctagaggacacaggattctcgttcgtgaagtgtaaggtgacagggacaggagtattgtaccttgggagggcatggggtcccttctcaagagtcgtatttgcttacacctatatggacaacatcatcctccctaaaggctggtacaattggggcgacccttcacgcgagatgacggtgttctatgggcagtacaagtgcacgggagcaggagcaaactatgcagggagggtggcttgggcaagagagctcaccgacgaagaagctaagccttttatatctcttaccttcatcgacggttctgaatggatcagactctaa

SEQ ID NO: 4 - protein, 382 aa, Brassica rapa
MPQFSSSQAPILILPVLIILLCSTQTQCHTKGLRLRPRNQKIVNSTSQTQNPEEEFLKWVRYVGSLKHTVFKAAKNKLFASYTLTVHKKHNKGDFTKIQDAIDSLPLINLVRVVIKVHAGVYKEKVNIPPMKAFITIEGEGADKTIVQWGDTAQTHDPKGNPMGTFNSASFAVNSPFFVAKNITFKNTTPVPLPGAVGKQAVALRVSADNAAFFGCKMLGAQDTLYDHLGRHYYKDCYIEGSVDFIFGNALSLYEGCHVHAIADKLGAVTAQGRSSVLEDTGFSFVKCKVTGTGVLYLGRAWGPFSRVVFAYTYMDNIILPKGWYNWGDPSREMTVFYGQYKCTGAGANYAGRVAWARELTDEEAKPFISLTFIDGSEWIRL

SEQ ID NO: 5 - DNA, 1065 bp, Solanum lycopersicum
atgttaatgttgtttactattagcacaagtagtgctagaagggataatacattgaaggtggctaatgaagaaaaagactacttgaattggattcatcgcatgagttctcgcaatcattctgttttccaagaagctaagaacaaattagagccttgtaaatttattaaggtgaataaaaacccgaaattcggagattttactacggttcagaaggctattgattcaatcccaatagtcaattcgtgtcgagtggttatttctgttagtcctggaacttacagggaaaagattgaaattccagcaacaatggcttacattaccctggaaggtgctgcttcacataaaacaactatcaaatgggatgacactgcagataggacaggaaaaagtggccaaccaatgggaacttatggttccgcaacttttgctgttaattccccctatttcattgccaaaaacatcacctttaagaatgtagcaccaccaccaccatcaggggcactaggaaagcaagcggtggcattaagaatatcggcagacacagcggcgttcataaattgcaagttcattggagcacaggacacactgtatgatcacaggggcaggcactatttcaagaactgttatattcaaggttctgtagattttatatttggtgatgggctctccctttatgagaattgtcatttacgtgcaaaaacaaaaagctatggggcattgacagcccagaagagggagagtttactggaggaaactggattctcttttctcaattgcaaagttactggatctggtgctctttacttgggcagggcttggggtactttctctagggtcgtatttgcttacacttatatggataaaattatcacatcaaagggatggtatgactggggagataagaacaggcatatgacggtattttttgggcaattcaagtgttcaggaccaggggcagaccatggtgaaagggtgaaatggtccagggagctcactgaacaagaagctaaaccgtttatctcactcagtttcatagatggtcatgaatggttactccatatttga

SEQ ID NO: 6 - protein, 354 aa, Solanum lycopersicum
MLMLFTISTSSARRDNTLKVANEEKDYLNWIHRMSSRNHSVFQEAKNKLEPCKFIKVNKNPKFGDFTTVQKAIDSIPIVNSCRVVISVSPGTYREKIEIPATMAYITLEGAASHKTTIKWDDTADRTGKSGQPMGTYGSATFAVNSPYFIAKNITFKNVAPPPPSGALGKQAVALRISADTAAFINCKFIGAQDTLYDHRGRHYFKNCYIQGSVDFIFGDGLSLYENCHLRAKTKSYGALTAQKRESLLEETGFSFLNCKVTGSGALYLGRAWGTFSRVVFAYTYMDKIITSKGWYDWGDKNRHMTVFFGQFKCSGPGADHGERVKWSRELTEQEAKPFISLSFIDGHEWLLHI

SEQ ID NO: 7 - DNA, 1155 bp, Oryza sativa
atggccgtggcgcccgtccggctcgtggcgtgcattgtcgccctggccgccgtggcgccgggcggagtggcggggcacacacggggcgtgcggccagggagggcggcggggaagcagcagccgtcgttcccggagaacgcgacgcgggtggaggcgatcgagcggcagttcatggagtgggtacggtacatgggcgggctggagcacagcacggtccaccacgcgctcgcccgggcgttcccctcctactcgctcgtcgtcgacaagaacccggcgttcggcgacttcaccaccatccaggccgccgtcgactcgctcccgatcatcaacctcgtccgcgtcgtcatcaaggtcaacgccggcacctacacggagaaggtgaacatatcgccgatgcgcgcgttcatcaccctcgagggcgccggcgccgacaagacgatcgtgcagtggggtgacaccgcggacagtccgtccggccgggcgggacggccgctcggcacatacagctccgcgtcgttcgccgtgaacgcgcagtacttcctcgccaggaacatcactttcaagaacacgtcgccggtgccgaagccgggggcgtcggggaagcaggcggtggcgctgcgggtgtcggcggacaacgcggcgttcgtggggtgcaggttcctgggcgcgcaggacacgctgtacgatcactcgggccggcactactacaaggaatgctacatcgaaggctccgtggatttcatctttggcaatgcgctctctctgtttgaggattgccacgtgcatgcgatcgcgcgggactacggcgcgctgacagcgcagaaccggcagagcatgctggaggacacggggttctcgttcgtcaactgccgggtgacgggatccggcgcgctctacctcggccgcgcctggggcaccttctcccgcgtcgtcttcgcctacacctacatggacgacatcatcatcccccgtggctggtacaactggggcgaccccaaccgcgagctgacggtgttctacgggcagtacaagtgcacgggccccggcgcgagcttctccggcagggtgtcgtggtcacgcgagctcaccgacgaggaggccaagcccttcatctcgctcaccttcatcgacggcacggaatgggtcaggttgtga

SEQ ID NO: 8 - protein, 384 aa, Oryza sativa
MAVAPVRLVACIVALAAVAPGGVAGHTRGVRPGRAAGKQQPSFPENATRVEAIERQFMEWVRYMGGLEHSTVHHALARAFPSYSLVVDKNPAFGDFTTIQAAVDSLPIINLVRVVIKVNAGTYTEKVNISPMRAFITLEGAGADKTIVQWGDTADSPSGRAGRPLGTYSSASFAVNAQYFLARNITFKNTSPVPKPGASGKQAVALRVSADNAAFVGCRFLGAQDTLYDHSGRHYYKECYIEGSVDFIFGNALSLFEDCHVHAIARDYGALTAQNRQSMLEDTGFSFVNCRVTGSGALYLGRAWGTFSRVVFAYTYMDDIIIPRGWYNWGDPNRELTVFYGQYKCTGPGASFSGRVSWSRELTDEEAKPFISLTFIDGTEWVRL

SEQ ID NO: 9 - DNA, 1011 bp, Oryza sativa
atggccgtggcgcccgtccggctcgtggcgtgcattgtcgccctggccgccgtggcgccgggcggagtggcggggcacacacggggcgtgcggccagggagggcggcggggaagcagcagccgtcgttcccggagaacgcgacgcgggtggaggcgatcgagcggcagttcatggagtgggtacggtacatgggcgggctggagcacagcacggtccaccacgcgctcgcccgggcgttcccctcctactcgctcgtcgtcgacaagaacccggcgttcggcgacttcaccaccatccaggccgccgtcgactcgctcccgatcatcaacctcgtccgcgtcgtcatcaaggtcaacgccggcacctacacggagaaggtgaacatatcgccgatgcgcgcgttcatcaccctcgagggcgccggcgccgacaagacgatcgtgcagtggggtgacaccgcggacagtccgtccggccgggcgggacggccgctcggcacatacagctccgcgtcgttcgccgtgaacgcgcagtacttcctcgccaggaacatcactttcaagaacacgtcgccggtgccgaagccgggggcgtcggggaagcaggcggtggcgctgcgggtgtcggcggacaacgcggcgttcgtggggtgcaggttcctgggcgcgcaggacacgctgtacgatcactcgggccggcactactacaaggaatgctacatcgaaggctccgtggatttcatctttggcaatgcgctctctctgtttgaggattgccacgtgcatgcgatcgcgcgggactacggcgcgctgacagcgcagaaccggcagagcatgctggaggacacggggttctcgttcgtcaactgccgggtgacgggatccggcgcgctctacctcggccgcgcctggggcaccttctcccgcgtcgtcttcgcctacacctacatggacgacatcatcatcccccgtggctggtacaactggggcgaccccaaccgcgagctgtaa

SEQ ID NO: 10 - protein, 336 aa, Oryza sativa
MAVAPVRLVACIVALAAVAPGGVAGHTRGVRPGRAAGKQQPSFPENATRVEAIERQFMEWVRYMGGLEHSTVHHALARAFPSYSLVVDKNPAFGDFTTIQAAVDSLPIINLVRVVIKVNAGTYTEKVNISPMRAFITLEGAGADKTIVQWGDTADSPSGRAGRPLGTYSSASFAVNAQYFLARNITFKNTSPVPKPGASGKQAVALRVSADNAAFVGCRFLGAQDTLYDHSGRHYYKECYIEGSVDFIFGNALSLFEDCHVHAIARDYGALTAQNRQSMLEDTGFSFVNCRVTGSGALYLGRAWGTFSRVVFAYTYMDDIIIPRGWYNWGDPNREL